European Patent Application EP 4 455 158 A1, published October 30, 2024. Title: CXCR3発現細胞遊走活性が増強したCXCR3リガンド。. Applicant: CHUGAI SEIYAKU KABUSHIKI KAISHA. The sequence listing filed with the application follows.

SEQUENCE LISTING (71 sequences)

SEQ ID NO: 1 - protein, 77 aa, synthetic construct
  source 1..77: note = An hCXCL10 variant hCXCL10R75A
VPLSRTVRCTCISISNQPVNPRSLEKLEIIPASQFCPRVEIIATMKKKGEKRCLNPESKAIKNLLKAVSKERSKASP

SEQ ID NO: 2 - protein, 230 aa, synthetic construct
  source 1..230: note = An hIgG1 Fc domain variant G1T4k.one
EPKSSDKTHTCPPCPAPELRRGPSVFLFPPKPKDTLMISRTPEVTCVVVDVSHEDPEVKFNWYVDGVEVHNAKTKPREEQYNSTYRVVSVLTVLHQDWLNGKEYKCKVSNKGLPSSIEKTISKAKGQPREPQVCTLPPSREEMTKNQVSLWCLVKGFYPSDIAVEWESNGQPENNYKTTPPVLDSDGSFFLYSKLTVDKSRWQEGNVFSCSVMHEALHNHYTQKSLSLSP

SEQ ID NO: 3 - protein, 230 aa, synthetic construct
  source 1..230: note = An hIgG1 Fc domain variant VHn-G1T4h.one.H435R
EPKSSDKTHTCPPCPAPELRRGPSVFLFPPKPKDTLMISRTPEVTCVVVDVSHEDPEVKFNWYVDGVEVHNAKTKPREEQYNSTYRVVSVLTVLHQDWLNGKEYKCKVSNKGLPSSIEKTISKAKGQPREPQVYTLPPSRCEMTKNQVSLSCAVKGFYPSDIAVEWESNGQPENNYKTTPPVLDSDGSFFLVSKLTVDKSRWQEGNVFSCSVMHEALHNRYTQKSLSLSP

SEQ ID NO: 4 - protein, 77 aa, synthetic construct
  source 1..77: note = An hCXCL10 variant hCXCL10R75A.0639
YPLSRTVRCTCISISNQPVNPRSLEKLEIIPASQFCPRVEIIATMKKKGEKRCLNPESKAIKNLLKAVSKERSKASP

SEQ ID NO: 5 - protein, 77 aa, synthetic construct
  source 1..77: note = An hCXCL10 variant hCXCL10R75A.0640
VPLSRTVRCTCISISNQCVNPRSLEKLEIIPASQFCPRVEIIATMKKKGEKRCLNPESKAIKNLLKAVSKERSKASP

SEQ ID NO: 6 - protein, 77 aa, synthetic construct
  source 1..77: note = An hCXCL10 variant hCXCL10R75A.0641
VPLSRTVRCTCISISNQPVNPRSLEKLEIIPASQFCPRVEIIATMKKKGEKRCLNPESKCIKNLLKAVSKERSKASP

SEQ ID NO: 7 - protein, 77 aa, synthetic construct
  source 1..77: note = An hCXCL10 variant hCXCL10R75A.0642
VPLSRTVRCTCISISNQCVNPRSLEKLEIIPASQFCPRVEIIATMKKKGEKRCLNPESKCIKNLLKAVSKERSKASP

SEQ ID NO: 8 - protein, 77 aa, synthetic construct
  source 1..77: note = An hCXCL10 variant hCXCL10R75A.0016
VVLSRTVRCTCISISNQPVNPRSLEKLEIIPASQFCPRVEIIATMKKKGEKRCLNPESKAIKNLLKAVSKERSKASP

SEQ ID NO: 9 - protein, 77 aa, synthetic construct
  source 1..77: note = An hCXCL10 variant hCXCL10R75A.0643
YVLSRTVRCTCISISNQPVNPRSLEKLEIIPASQFCPRVEIIATMKKKGEKRCLNPESKAIKNLLKAVSKERSKASP

SEQ ID NO: 10 - protein, 77 aa, synthetic construct
  source 1..77: note = An hCXCL10 variant hCXCL10R75A.0644
VVLSRTVRCTCISISNQCVNPRSLEKLEIIPASQFCPRVEIIATMKKKGEKRCLNPESKCIKNLLKAVSKERSKASP

SEQ ID NO: 11 - protein, 77 aa, synthetic construct
  source 1..77: note = An hCXCL10 variant hCXCL10R75A.0669
YPLSRTVRCTCISISNQCVNPRSLEKLEIIPASQFCPRVEIIATMKKKGEKRCLNPESKCIKNLLKAVSKERSKASP

SEQ ID NO: 12 - protein, 77 aa, synthetic construct
  source 1..77: note = An hCXCL10 variant hCXCL10R75A.0670
YVLSRTVRCTCISISNQCVNPRSLEKLEIIPASQFCPRVEIIATMKKKGEKRCLNPESKCIKNLLKAVSKERSKASP

SEQ ID NO: 13 - protein, 6 aa, synthetic construct
  source 1..6: note = An N-terminal sequence of a CXCR3 ligand
YPLSRT

SEQ ID NO: 14 - protein, 6 aa, synthetic construct
  source 1..6: note = An N-terminal sequence of a CXCR3 ligand
YVLSRT

SEQ ID NO: 15 - protein, 8 aa, synthetic construct
  source 1..8: note = An N-terminal sequence of a CXCR3 ligand
YPLSRTVR

SEQ ID NO: 16 - protein, 8 aa, synthetic construct
  source 1..8: note = An N-terminal sequence of a CXCR3 ligand
YVLSRTVR

SEQ ID NO: 17-18 - skipped (2 entries)

SEQ ID NO: 19 - protein, 6 aa, synthetic construct
  source 1..6: note = An N-terminal sequence of a parent CXCR3 ligand
VPLSRT

SEQ ID NO: 20 - protein, 6 aa, synthetic construct
  source 1..6: note = An N-terminal sequence of a parent CXCR3 ligand
VVLSRT

SEQ ID NO: 21 - protein, 8 aa, synthetic construct
  source 1..8: note = An N-terminal sequence of a parent CXCR3 ligand
VPLSRTVR

SEQ ID NO: 22 - protein, 8 aa, synthetic construct
  source 1..8: note = An N-terminal sequence of a parent CXCR3 ligand
VVLSRTVR

SEQ ID NO: 23-24 - skipped (2 entries)

SEQ ID NO: 25 - protein, 77 aa, Homo sapiens
  source 1..77: note = hCXCL10
VPLSRTVRCTCISISNQPVNPRSLEKLEIIPASQFCPRVEIIATMKKKGEKRCLNPESKAIKNLLKAVSKERSKRSP

SEQ ID NO: 26 - protein, 73 aa, Homo sapiens
  source 1..73: note = hCXCL11
FPMFKRGRCLCIGPGVKAVKVADIEKASIMYPSNNCDKIEVIITLKENKGQRCLNPKSKQARLIIKKVERKNF

SEQ ID NO: 27 - protein, 103 aa, Homo sapiens
  source 1..103: note = hCXCL9
TPVVRKGRCSCISTNQGTIHLQSLKDLKQFAPSPSCEKIEIIATLKNGVQTCLNPDSADVKELIKKWEKQVSQKKKQKNGKKHQKKKVLKVRKSQRSRQKKTT

SEQ ID NO: 28 - protein, 77 aa, synthetic construct
  source 1..77: note = An hCXCL11-hCXCL10 chimeric protein
FPMFKRGRCLCIGPGVKAVKVADIEKLEIIPASQFCPRVEIIATMKKKGEKRCLNPESKAIKNLLKAVSKERSKASP

SEQ ID NO: 29 - protein, 4 aa, synthetic construct
  source 1..4: note = An artificially synthesized linker sequence
GGGS

SEQ ID NO: 30 - protein, 4 aa, synthetic construct
  source 1..4: note = An artificially synthesized linker sequence
GGSG

SEQ ID NO: 31 - protein, 4 aa, synthetic construct
  source 1..4: note = An artificially synthesized linker sequence
GSGG

SEQ ID NO: 32 - protein, 4 aa, synthetic construct
  source 1..4: note = An artificially synthesized linker sequence
SGGG

SEQ ID NO: 33 - protein, 4 aa, synthetic construct
  source 1..4: note = An artificially synthesized linker sequence
GSSG

SEQ ID NO: 34 - protein, 5 aa, synthetic construct
  source 1..5: note = An artificially synthesized linker sequence
GGGGS

SEQ ID NO: 35 - protein, 5 aa, synthetic construct
  source 1..5: note = An artificially synthesized linker sequence
GGGSG

SEQ ID NO: 36 - protein, 5 aa, synthetic construct
  source 1..5: note = An artificially synthesized linker sequence
GGSGG

SEQ ID NO: 37 - protein, 5 aa, synthetic construct
  source 1..5: note = An artificially synthesized linker sequence
GSGGG

SEQ ID NO: 38 - protein, 5 aa, synthetic construct
  source 1..5: note = An artificially synthesized linker sequence
GSGGS

SEQ ID NO: 39 - protein, 5 aa, synthetic construct
  source 1..5: note = An artificially synthesized linker sequence
SGGGG

SEQ ID NO: 40 - protein, 5 aa, synthetic construct
  source 1..5: note = An artificially synthesized linker sequence
GSSGG

SEQ ID NO: 41 - protein, 5 aa, synthetic construct
  source 1..5: note = An artificially synthesized linker sequence
GSGSG

SEQ ID NO: 42 - protein, 5 aa, synthetic construct
  source 1..5: note = An artificially synthesized linker sequence
SGGSG

SEQ ID NO: 43 - protein, 5 aa, synthetic construct
  source 1..5: note = An artificially synthesized linker sequence
GSSSG

SEQ ID NO: 44 - protein, 6 aa, synthetic construct
  source 1..6: note = An artificially synthesized linker sequence
GGGGGS

SEQ ID NO: 45 - protein, 6 aa, synthetic construct
  source 1..6: note = An artificially synthesized linker sequence
SGGGGG

SEQ ID NO: 46 - protein, 7 aa, synthetic construct
  source 1..7: note = An artificially synthesized linker sequence
GGGGGGS

SEQ ID NO: 47 - protein, 7 aa, synthetic construct
  source 1..7: note = An artificially synthesized linker sequence
SGGGGGG

SEQ ID NO: 48 - protein, 21 aa, synthetic construct
  source 1..21: note = A signal sequence derived from human CXCL10
MNQTAILICCLIFLTLSGIQG

SEQ ID NO: 49 - protein, 22 aa, synthetic construct
  source 1..22: note = A signal sequence derived from human CXCL9
MKKSGVLFLLGIILLVLIGVQG

SEQ ID NO: 50 - protein, 21 aa, synthetic construct
  source 1..21: note = A signal sequence derived from human CXCL11
MSVKGMAIALAVILCATVVQG

SEQ ID NO: 51 - protein, 368 aa, Homo sapiens
  source 1..368: note = hCXCR3
MVLEVSDHQVLNDAEVAALLENFSSSYDYGENESDSCCTSPPCPQDFSLNFDRAFLPALYSLLFLLGLLGNGAVAAVLLSRRTALSSTDTFLLHLAVADTLLVLTLPLWAVDAAVQWVFGSGLCKVAGALFNINFYAGALLLACISFDRYLNIVHATQLYRRGPPARVTLTCLAVWGLCLLFALPDFIFLSAHHDERLNATHCQYNFPQVGRTALRVLQLVAGFLLPLLVMAYCYAHILAVLLVSRGQRRLRAMRLVVVVVVAFALCWTPYHLVVLVDILMDLGALARNCGRESRVDVAKSVTSGLGYMHCCLNPLLYAFVGVKFRERMWMLLLRLGCPNQRGLQRQPSSSRRDSSWSETSEASYSGL

SEQ ID NO: 52 - protein, 19 aa, synthetic construct
  source 1..19: note = A signal sequence
MGWSCIILFLVATATGVHS

SEQ ID NO: 53 - protein, 77 aa, synthetic construct
  SITE 1: note = X = Val or Tyr
  SITE 2: note = X = Pro or Val
  SITE 18: note = X = Cys
  SITE 60: note = X = Cys
  SITE 75: note = X = Arg or Ala
  source 1..77: note = An artificially synthesized polypeptide sequence
XXLSRTVRCTCISISNQXVNPRSLEKLEIIPASQFCPRVEIIATMKKKGEKRCLNPESKXIKNLLKAVSKERSKXSP

SEQ ID NO: 54 - protein, 77 aa, synthetic construct; identical to SEQ ID NO: 53
  SITE 1: note = X = Tyr
  SITE 2: note = X = Pro or Val
  SITE 18: note = X = Pro or Cys
  SITE 60: note = X = Ala or Cys
  SITE 75: note = X = Arg or Ala
  source 1..77: note = An artificially synthesized polypeptide sequence

SEQ ID NO: 55 - protein, 77 aa, synthetic construct
  source 1..77: note = An hCXCL10 variant hCXCL10R75A.0303
VVLSRTPRCTCISISNQPVNPRSLEKLEIIPASQFCPRVEIIATMKKKGEKRCLNPESKAIKNLLKAVSKERSKASP

SEQ ID NO: 56 - protein, 462 aa, synthetic construct
  source 1..462: note = An antibody heavy chain G7HFR0039H-G1T4h
QVQLVESGGGVVQPGRSLRLSCAASGFTFSSFSITWIRQPPGKGLEWIGEITPMFGIANYAQKFQGQVTISADKSISTAYLQWSSLKASDTAMYYCARDGRFDVSDLLTDKPKVTINYNGMDVWGQGTLVTVSSASTKGPSVFPLAPSSKSTSGGTAALGCLVKDYFPEPVTVSWNSGALTSGVHTFPAVLQSSGLYSLSSVVTVPSSSLGTQTYICNVNHKPSNTKVDKRVEPKSCDKTHTCPPCPAPELRRGPSVFLFPPKPKDTLMISRTPEVTCVVVDVSHEDPEVKFNWYVDGVEVHNAKTKPREEQYNSTYRVVSVLTVLHQDWLNGKEYKCKVSNKGLPSSIEKTISKAKGQPREPQVYTLPPSRCEMTKNQVSLSCAVKGFYPSDIAVEWESNGQPENNYKTTPPVLDSDGSFFLVSKLTVDKSRWQEGNVFSCSVMHEALHNHYTQKSLSLSP

SEQ ID NO: 57 - protein, 216 aa, synthetic construct
  source 1..216: note = An antibody light chain G7L-LT0
QSVLTQPPSASGTPGQRVTISCSGSSSNIGSNTVNWYQRLPGAAPQLLIYNNDQRPSGIPDRFSGSKSGTSGSLVISGLQSEDEADYYCASWDDSLNGRVFGGGTKLTVLGQPKAAPSVTLFPPSSEELQANKATLVCLISDFYPGAVTVAWKADSSPVKAGVETTTPSKQSNNKYAASSYLSLTPEQWKSHRSYSCQVTHEGSTVEKTVAPTECS

SEQ ID NO: 58 - protein, 474 aa, synthetic construct
  source 1..474: note = An antibody heavy chain G7HFR0039H.12aa0054-G1T4h
QVQLVESGGGVVQPGRSLRLSCAASGFTFSSFSITWIRQPPGKGLEWIGEITPMFGIANYAQKFQGQVTISADKSISTAYLQWSSLKASDTAMYYCARDGRFDVSDLLTDKPKVTINYNGMDVWGQGTLVTVSSTSGSGRSATPRGASTKGPSVFPLAPSSKSTSGGTAALGCLVKDYFPEPVTVSWNSGALTSGVHTFPAVLQSSGLYSLSSVVTVPSSSLGTQTYICNVNHKPSNTKVDKRVEPKSCDKTHTCPPCPAPELRRGPSVFLFPPKPKDTLMISRTPEVTCVVVDVSHEDPEVKFNWYVDGVEVHNAKTKPREEQYNSTYRVVSVLTVLHQDWLNGKEYKCKVSNKGLPSSIEKTISKAKGQPREPQVYTLPPSRCEMTKNQVSLSCAVKGFYPSDIAVEWESNGQPENNYKTTPPVLDSDGSFFLVSKLTVDKSRWQEGNVFSCSVMHEALHNHYTQKSLSLSP

SEQ ID NO: 59 - protein, 560 aa, synthetic construct
  source 1..560: note = An hCXCL10 variant-antibody heavy chain fusion protein hCXCL10R75A.G4SGGGG.G7HFR0039H.12aa0054-G1T4h
VPLSRTVRCTCISISNQPVNPRSLEKLEIIPASQFCPRVEIIATMKKKGEKRCLNPESKAIKNLLKAVSKERSKASPGGGGSGGGGQVQLVESGGGVVQPGRSLRLSCAASGFTFSSFSITWIRQPPGKGLEWIGEITPMFGIANYAQKFQGQVTISADKSISTAYLQWSSLKASDTAMYYCARDGRFDVSDLLTDKPKVTINYNGMDVWGQGTLVTVSSTSGSGRSATPRGASTKGPSVFPLAPSSKSTSGGTAALGCLVKDYFPEPVTVSWNSGALTSGVHTFPAVLQSSGLYSLSSVVTVPSSSLGTQTYICNVNHKPSNTKVDKRVEPKSCDKTHTCPPCPAPELRRGPSVFLFPPKPKDTLMISRTPEVTCVVVDVSHEDPEVKFNWYVDGVEVHNAKTKPREEQYNSTYRVVSVLTVLHQDWLNGKEYKCKVSNKGLPSSIEKTISKAKGQPREPQVYTLPPSRCEMTKNQVSLSCAVKGFYPSDIAVEWESNGQPENNYKTTPPVLDSDGSFFLVSKLTVDKSRWQEGNVFSCSVMHEALHNHYTQKSLSLSP

SEQ ID NO: 60 - protein, 560 aa, synthetic construct
  source 1..560: note = An hCXCL10 variant-antibody heavy chain fusion protein hCXCL10R75A.0016.G4SGGGG.G7HFR0039H.12aa0054-G1T4h
VVLSRTVRCTCISISNQPVNPRSLEKLEIIPASQFCPRVEIIATMKKKGEKRCLNPESKAIKNLLKAVSKERSKASPGGGGSGGGGQVQLVESGGGVVQPGRSLRLSCAASGFTFSSFSITWIRQPPGKGLEWIGEITPMFGIANYAQKFQGQVTISADKSISTAYLQWSSLKASDTAMYYCARDGRFDVSDLLTDKPKVTINYNGMDVWGQGTLVTVSSTSGSGRSATPRGASTKGPSVFPLAPSSKSTSGGTAALGCLVKDYFPEPVTVSWNSGALTSGVHTFPAVLQSSGLYSLSSVVTVPSSSLGTQTYICNVNHKPSNTKVDKRVEPKSCDKTHTCPPCPAPELRRGPSVFLFPPKPKDTLMISRTPEVTCVVVDVSHEDPEVKFNWYVDGVEVHNAKTKPREEQYNSTYRVVSVLTVLHQDWLNGKEYKCKVSNKGLPSSIEKTISKAKGQPREPQVYTLPPSRCEMTKNQVSLSCAVKGFYPSDIAVEWESNGQPENNYKTTPPVLDSDGSFFLVSKLTVDKSRWQEGNVFSCSVMHEALHNHYTQKSLSLSP

SEQ ID NO: 61 - protein, 560 aa, synthetic construct
  source 1..560: note = An hCXCL10 variant-antibody heavy chain fusion protein hCXCL10R75A.0303.G4SGGGG.G7HFR0039H.12aa0054-G1T4h
VVLSRTPRCTCISISNQPVNPRSLEKLEIIPASQFCPRVEIIATMKKKGEKRCLNPESKAIKNLLKAVSKERSKASPGGGGSGGGGQVQLVESGGGVVQPGRSLRLSCAASGFTFSSFSITWIRQPPGKGLEWIGEITPMFGIANYAQKFQGQVTISADKSISTAYLQWSSLKASDTAMYYCARDGRFDVSDLLTDKPKVTINYNGMDVWGQGTLVTVSSTSGSGRSATPRGASTKGPSVFPLAPSSKSTSGGTAALGCLVKDYFPEPVTVSWNSGALTSGVHTFPAVLQSSGLYSLSSVVTVPSSSLGTQTYICNVNHKPSNTKVDKRVEPKSCDKTHTCPPCPAPELRRGPSVFLFPPKPKDTLMISRTPEVTCVVVDVSHEDPEVKFNWYVDGVEVHNAKTKPREEQYNSTYRVVSVLTVLHQDWLNGKEYKCKVSNKGLPSSIEKTISKAKGQPREPQVYTLPPSRCEMTKNQVSLSCAVKGFYPSDIAVEWESNGQPENNYKTTPPVLDSDGSFFLVSKLTVDKSRWQEGNVFSCSVMHEALHNHYTQKSLSLSP

SEQ ID NO: 62 - protein, 444 aa, synthetic construct
  source 1..444: note = An antibody heavy chain IC17HdK-G1T4k.H435R
QVQLQQSGPQLVRPGASVKISCKASGYSFTSYWMHWVNQRPGQGLEWIGMIDPSYSETRLNQKFKDKATLTVDKSSSTAYMQLSSPTSEDSAVYYCALYGNYFDYWGQGTTLTVSSASTKGPSVFPLAPSSKSTSGGTAALGCLVKDYFPEPVTVSWNSGALTSGVHTFPAVLQSSGLYSLSSVVTVPSSSLGTQTYICNVNHKPSNTKVDKRVEPKSCDKTHTCPPCPAPELRRGPSVFLFPPKPKDTLMISRTPEVTCVVVDVSHEDPEVKFNWYVDGVEVHNAKTKPREEQYNSTYRVVSVLTVLHQDWLNGKEYKCKVSNKGLPSSIEKTISKAKGQPREPQVCTLPPSREEMTKNQVSLWCLVKGFYPSDIAVEWESNGQPENNYKTTPPVLDSDGSFFLYSKLTVDKSRWQEGNVFSCSVMHEALHNRYTQKSLSLSP

SEQ ID NO: 63 - protein, 77 aa, synthetic construct
  source 1..77: note = An hCXCL10 variant hCXCL10R75A.0613
YVLSRTPRCTCISISNQCVNPRSLEKLEIIPASQFCPRVEIIATMKKKGEKRCLNPESKCIKNLLKAVSKERSKASP

SEQ ID NO: 64 - protein, 560 aa, synthetic construct
  source 1..560: note = An hCXCL10 variant-antibody heavy chain fusion protein hCXCL10R75A.0659.G4SGGGG.G7HFR0039H.0004.N0222-G1T4h
VVLSRTPRCTCISISNQCVNPRSLEKLEIIPASQFCPRVEIIATMKKKGEKRCLNPESKCIKNLLKAVSKERSKASPGGGGSGGGGQVQLVESGGGVVQPGRSLRLSCAASGFTFSSFSITWIRDPPGKGLEWIGEITPMFGIAFYAQKFQGQVTISADKSISTAYLQWSSLKASDTAMYYCARDGRFDVSDLLTDKPKVTINYNGMDVWGQGTLVTVSSYSATGRSANPRGASTKGPSVFPLAPSSKSTSGGTAALGCLVKDYFPEPVTVSWNSGALTSGVHTFPAVLQSSGLYSLSSVVTVPSSSLGTQTYICNVNHKPSNTKVDKRVEPKSCDKTHTCPPCPAPELRRGPSVFLFPPKPKDTLMISRTPEVTCVVVDVSHEDPEVKFNWYVDGVEVHNAKTKPREEQYNSTYRVVSVLTVLHQDWLNGKEYKCKVSNKGLPSSIEKTISKAKGQPREPQVYTLPPSRCEMTKNQVSLSCAVKGFYPSDIAVEWESNGQPENNYKTTPPVLDSDGSFFLVSKLTVDKSRWQEGNVFSCSVMHEALHNHYTQKSLSLSP

SEQ ID NO: 65 - protein, 216 aa, synthetic construct
  source 1..216: note = An antibody light chain G7L.R38E-LT0
QSVLTQPPSASGTPGQRVTISCSGSSSNIGSNTVNWYQELPGAAPQLLIYNNDQRPSGIPDRFSGSKSGTSGSLVISGLQSEDEADYYCASWDDSLNGRVFGGGTKLTVLGQPKAAPSVTLFPPSSEELQANKATLVCLISDFYPGAVTVAWKADSSPVKAGVETTTPSKQSNNKYAASSYLSLTPEQWKSHRSYSCQVTHEGSTVEKTVAPTECS

SEQ ID NO: 66 - protein, 9 aa, synthetic construct
  source 1..9: note = An artificially synthesized linker sequence
GGGGSGGGG

SEQ ID NO: 67 - protein, 7 aa, synthetic construct
  source 1..7: note = An N-terminal sequence of a CXCR3 ligand
YPLSRTP

SEQ ID NO: 68 - protein, 7 aa, synthetic construct
  source 1..7: note = An N-terminal sequence of a CXCR3 ligand
YVLSRTP

SEQ ID NO: 69 - protein, 77 aa, synthetic construct
  source 1..77: note = An artificially synthesized polypeptide sequence
  SITE 1: note = X = Val or Tyr
  SITE 2: note = X = Pro or Val
  SITE 7: note = X = Pro
  SITE 18: note = X = Pro or Cys
  SITE 60: note = X = Ala or Cys
  SITE 75: note = X = Arg or Ala
XXLSRTXRCTCISISNQXVNPRSLEKLEIIPASQFCPRVEIIATMKKKGEKRCLNPESKXIKNLLKAVSKERSKXSP

SEQ ID NO: 70 - protein, 7 aa, synthetic construct
  source 1..7: note = An N-terminal sequence of a CXCR3 ligand
VPLSRTP

SEQ ID NO: 71 - protein, 7 aa, synthetic construct
  source 1..7: note = An N-terminal sequence of a CXCR3 ligand
VVLSRTP